European Patent Application EP 4 660 317 A1, published December 10, 2025. Title: Method for barcoding molecules in single-cell experiments. Applicant: Miltenyi Biotec BV Co KG. Application EP MBG_168, filed June 5, 2024. The sequence listing filed with the application follows.

SEQUENCE LISTING (7 sequences)

SEQ ID NO: 1 - DNA, 78 bp, synthetic construct
  source 1..78: mol_type = other DNA
aatgatacggcgaccaccgagatctacacnnnnnnnnnnnnnnnnacactctttccctacacgacgctcttccgatct

SEQ ID NO: 2 - DNA, 50 bp, synthetic construct
  source 1..50: mol_type = other DNA
ctacacgacgctcttccgatctnnnnnnnnnnnntttcttatatrgrgrg

SEQ ID NO: 3 - DNA, 57 bp, synthetic construct
  source 1..57: mol_type = other DNA
aagcagtggtatcaacgcagagtacttttttttttttttttttttttttttttttvn

SEQ ID NO: 4 - DNA, 27 bp, synthetic construct
  source 1..27: mol_type = other DNA
aatgatacggcgaccaccgagatctac

SEQ ID NO: 5 - DNA, 24 bp, synthetic construct
  source 1..24: mol_type = other DNA
gaagagcgtcgtgtagggaaagag

SEQ ID NO: 6 - DNA, 23 bp, synthetic construct
  source 1..23: mol_type = other DNA
ctttccctacacgacgctcttcc

SEQ ID NO: 7 - DNA, 25 bp, synthetic construct
  source 1..25: mol_type = other DNA
aagcagtggtatcaacgcagagtac